European Patent Specification EP 3 821 011 B1, published April 26, 2023. Title: TRANSPOSOME ENABLED DNA/RNA-SEQUENCING (TED RNA-SEQ). Applicant: X GEN US CO. The sequence listing filed with the application follows.

SEQUENCE LISTING (3 sequences)

SEQ ID NO: 1 - DNA, 46 bp, Artificial Sequence
  Description of Artificial Sequence: Synthetic oligonucleotide
gtaggtgtgagtgatggttgaggtagtagatgtgtataagagacag

SEQ ID NO: 2 - DNA, 19 bp, Artificial Sequence
  Description of Artificial Sequence: Synthetic oligonucleotide
ctgtctcttatacacatct

SEQ ID NO: 3 - DNA, 46 bp, Artificial Sequence
  Description of Artificial Sequence: Synthetic oligonucleotide
gtgagtgatggttgaggtagtgtggagagatgtgtataagagacag